European Patent Application EP 4 154 878 A1, published March 29, 2023. Title: APPLICATION OF THE ACTIVE INGREDIENT OF SALVIA MILTIORRHIZA OR ITS PHARMACEUTICALLY ACCEPTABLE SALT IN THE PREPARATION OF ANTI-SARS-COV-2 DRUGS. Applicant: SOUTHERN MEDICAL UNIVERSITY. The sequence listing filed with the application follows.

SEQUENCE LISTING (4 sequences)

SEQ ID NO: 1 - DNA, 21 bp, Artificial Sequence
caatggtttaacaggcacagg

SEQ ID NO: 2 - DNA, 21 bp, Artificial Sequence
ctcaagtgtctgtggatcacg

SEQ ID NO: 3 - protein, 42 aa, Artificial Sequence
ANQFNSAIGKIQDSLSSTASALGKLQDVVNQNAQALNTLVKQ

SEQ ID NO: 4 - protein, 36 aa, Artificial Sequence
DISGINASVVNIQKEIDRLNEVAKNLNESLIDLQEL